European Patent Specification EP 3 323 831 B1, published April 12, 2023. Title: Aggrus monoclonal antibody. Applicant: Japanese Foundation for Cancer Research. The sequence listing filed with the application follows.

SEQUENCE LISTING (19 sequences)

SEQ ID NO: 1 - protein, 9 aa, Homo sapiens
GIRIEDLPT

SEQ ID NO: 2 - protein, 17 aa, Homo sapiens
GAEDDVVTPGTSEDRYK

SEQ ID NO: 3 - protein, 5 aa, Homo sapiens
RIEDL

SEQ ID NO: 4 - protein, 6 aa, Homo sapiens
  misc_feature (3)..(4): Xaa can be any naturally occurring amino acid
EDXXTS

SEQ ID NO: 5 - protein, 144 aa, Homo sapiens
MWKVSALLFVLGSASLWVLAEGASTGQPEDDTETTGLEGGVAMPGAEDDVVTPGTSEDRYKSGLTTLVATSVNSVTGIRIEDLPTSESTVHAQEQSPSATASNVATSHSTEKVDGDTQTTVEKDGLSTVTLVGIIVGVLLAIGF

SEQ ID NO: 6 - protein, 144 aa, Pan paniscus
MWKVSALLFVLGSASLWVLAEGASTGQPEDDTETTGLEGGFAVPGAEDDVVTPGTSEDRYKSGLTTLVATSVNSVTGIRIEDLPTSESTVHAQEQSPSATASNVATSHSTEKVDGDTQTTVEKDGLATVTLVGIIVGVLLAIGF

SEQ ID NO: 7 - protein, 144 aa, Macaca mulatta
MWKVSALLFVLGSASLWVLAEGASTGQPEDDIETTGMEGGVAMPGAEDDVVTPGTSEDRYKSGLTTPVATSVNSVTDIHIEDLPTPESTVHAQGQSPSTTASNVATSHSTDKVDGDTQTAIEKDGLATVTLVGIIVGVLLAIGF

SEQ ID NO: 8 - protein, 141 aa, Sus scrofa
MWKVPVLLFVLGSASLWVLAEGASTVLPEDGVTPGVEGSSKASPGVEDYTVTPRTREEPYATPLVPTRTKGTTGSPTEDVFTVGSTTHSHKGSQSTTTQNVVTSQSHDKGDEEKSKTVTKDGLGTVTLVGITVGVLLAIGF

SEQ ID NO: 9 - protein, 143 aa, Physeter catodon
MWKGPVLFFVLGSASLWVLAEASTVRPEDGMTTGVENGKATPGVEDHVETPGASGEPHESAGLTAPMPTRTKSMTEVHKEDLPTAESTIHSQGQSQSTTTLNVATSQSPGKTDGEKPTTVEKGGSSTVTLVGIIVGVLLAIGF

SEQ ID NO: 10 - protein, 152 aa, Bos taurus
MWKVPVLFFILGSASFWVLAEGASTVRPEDDVTTGVTSEKTTLGVEDYTTTPAASKESLATPMPAGTENVSHDHREDLPTAEGTTAEGTTAKSTPARSTPARSTTTVLTRVPATSHSQGKTDGEKPKSTQKGGLSVGTLVGIIVGVLVGIAV

SEQ ID NO: 11 - protein, 151 aa, Canis lupus
MWRVPVLLLVLGGAGLRVPAAGASTVRPDDIIPGVEDSVVTPGTEDSVVTPGAEDNVVTDGATEEPYESGLTPLVTKNTESVTDLHLEDGPTQESTVHAKEESQSTTTLNVVTSHSREKVGEDTETTVEKDGLATVTLVGIIVGVLLAIGF

SEQ ID NO: 12 - protein, 140 aa, Myotis brandtii
MWKARVLLLVWGSALLWAPAGGASTVLPEDEATTASMENGMVTPGVGGNTMTPGASEQSHKPVGFTSQVPTNTKRTDTPIEDLPTTESTGHAQEETQSTTALNGATSHPREDTQTTGAKDGFSTGTLIGIIVGVLLGIGF

SEQ ID NO: 13 - protein, 148 aa, Rattus norvegicus
MWTAPVLLWVLGSVWFWDSAQGGAIGALEDDLVTPGPGDDMVNPGLEDRIETTDTTGELDKSTAKAPLVPTQPPIEELPTSGTSDHDHKEHESTTTVKAVTSHSTDKKTTHSNRDNAGGETQTTDKKDGLAVVTLVGIIIGVLLAIGF

SEQ ID NO: 14 - protein, 154 aa, Mus musculus
MWTVPVLFWVLGSVWFWDSAQGGTIGVNEDDIVTPGTGDGMVPPGIEDKITTTGATGGLNESTGKAPLVPTQRERGTKPPLEELSTSATSDHDHREHESTTTVKVVTSHSVDKKTSHPNRDNAGDETQTTDKKDGLPVVTLVGIIVGVLLAIGF

SEQ ID NO: 15 - protein, 8 aa, Homo sapiens
  misc_feature (3)..(4): Xaa can be any naturally occurring amino acid
EDXXVTPG

SEQ ID NO: 16 - protein, 8 aa, Homo sapiens
EDDTETTG

SEQ ID NO: 17 - protein, 8 aa, Homo sapiens
EGGVAMPG

SEQ ID NO: 18 - protein, 8 aa, Homo sapiens
EDDVVTPG

SEQ ID NO: 19 - protein, 7 aa, Homo sapiens
EDLPTSE